European Patent Application EP 4 219 756 A1, published August 2, 2023. Title: SYNTHETIC RNA FRAGMENT AND ITS USES FOR RNA-DEPENDENT AMPLIFICATION. Applicant: MELLO BIOTECH TAIWAN CO., LTD. Application EP. The sequence listing filed with the application follows.

SEQUENCE LISTING (4 sequences)

SEQ ID NO: 1 - DNA, 48 bp, synthetic construct
  source 1..48: mol_type = other DNA
gatatctaatacgactcactatagggagaggtatggtacttggtagtt

SEQ ID NO: 2 - DNA, 23 bp, synthetic construct
  source 1..23: mol_type = other DNA
gacaacaggtgcgctcaggtcct

SEQ ID NO: 3 - DNA, 56 bp, synthetic construct
  source 1..56: mol_type = other DNA
gatatctaatacgactcactatagggagatctgtgggaactagttcaggaaggtaa

SEQ ID NO: 4 - DNA, 32 bp, synthetic construct
  source 1..32: mol_type = other DNA
gttctcctaagcctgtagccaagaactgcaca